European Patent Application EP 4 592 322 A1, published July 30, 2025. Title: FUSION PROTEIN TARGETING INTERGRIN ALPHA(IIB)BETA3 AND CONTAINING TISSUE PLASMINOGEN ACTIVATOR OR VARIANT THEREOF AND USE THEREOF. Applicant: WOEI-JER CHUANG. Application EP. The sequence listing filed with the application follows.

SEQUENCE LISTING (42 sequences)

SEQ ID NO: 1 - protein, 9 aa, synthetic construct
GGGGGGGGG

SEQ ID NO: 2 - protein, 15 aa, synthetic construct
GGGGSGGGGSGGGGS

SEQ ID NO: 3 - protein, 6 aa, synthetic construct
PAPAPA

SEQ ID NO: 4 - protein, 10 aa, synthetic construct
PAPAPAPAPA

SEQ ID NO: 5 - protein, 14 aa, synthetic construct
PAPAPAPAPAPAPA

SEQ ID NO: 6 - protein, 15 aa, synthetic construct
EAAAKGGGGSGGGGS

SEQ ID NO: 7 - protein, 15 aa, synthetic construct
EAAAKEAAAKEAAAK

SEQ ID NO: 8 - protein, 527 aa, synthetic construct
SYQVICRDEKTQMIYQQHQSWLRPVLRSNRVEYCWCNSGRAQCHSVPVKSCSEPRCFNGGTCQQALYFSDFVCQCPEGFAGKCCEIDTRATCYEDQGISYRGTWSTAESGAECTNWNSSALAQKPYSGRRPDAIRLGLGNHNYCRNPDRDSKPWCYVFKAGKYSSEFCSTPACSEGNSDCYFGNGSAYRGTHSLTESGASCLPWNSMILIGKVYTAQNPSAQALGLGKHNYCRNPDGDAKPWCHVLKNRRLTWEYCDVPSCSTCGLRQYSQPQFRIKGGLFADIASHPWQAAIFAKHRRSPGERFLCGGILISSCWILSAAHCFQERFPPHHLTVILGRTYRVVPGEEEQKFEVEKYIVHKEFDDDTYDNDIALLQLKSDSSRCAQESSVVRTVCLPPADLQLPDWTECELSGYGKHEALSPFYSERLKEAHVRLYPSSRCTSQHLLNRTVTDNMLCAGDTRSGGPQANLHDACQGDSGGPLVCLNDGRMTLVGIISWGLGCGQKDVPGVYTKVTNYLDWIRDNMRP

SEQ ID NO: 9 - protein, 355 aa, synthetic construct
SYQGNSDCYFGNGSAYRGTHSLTESGASCLPWNSMILIGKVYTAQNPSAQALGLGKHNYCRNPDGDAKPWCHVLKNRRLTWEYCDVPSCSTCGLRQYSQPQFRIKGGLFADIASHPWQAAIFAKHRRSPGERFLCGGILISSCWILSAAHCFQERFPPHHLTVILGRTYRVVPGEEEQKFEVEKYIVHKEFDDDTYDNDIALLQLKSDSSRCAQESSVVRTVCLPPADLQLPDWTECELSGYGKHEALSPFYSERLKEAHVRLYPSSRCTSQHLLNRTVTDNMLCAGDTRSGGPQANLHDACQGDSGGPLVCLNDGRMTLVGIISWGLGCGQKDVPGVYTKVTNYLDWIRDNMRP

SEQ ID NO: 10 - protein, 527 aa, synthetic construct
SYQVICRDEKTQMIYQQHQSWLRPVLRSNRVEYCWCNSGRAQCHSVPVKSCSEPRCFNGGTCQQALYFSDFVCQCPEGFAGKCCEIDTRATCYEDQGISYRGNWSTAESGAECTNWQSSALAQKPYSGRRPDAIRLGLGNHNYCRNPDRDSKPWCYVFKAGKYSSEFCSTPACSEGNSDCYFGNGSAYRGTHSLTESGASCLPWNSMILIGKVYTAQNPSAQALGLGKHNYCRNPDGDAKPWCHVLKNRRLTWEYCDVPSCSTCGLRQYSQPQFRIKGGLFADIASHPWQAAIFAAAAASPGERFLCGGILISSCWILSAAHCFQERFPPHHLTVILGRTYRVVPGEEEQKFEVEKYIVHKEFDDDTYDNDIALLQLKSDSSRCAQESSVVRTVCLPPADLQLPDWTECELSGYGKHEALSPFYSERLKEAHVRLYPSSRCTSQHLLNRTVTDNMLCAGDTRSGGPQANLHDACQGDSGGPLVCLNDGRMTLVGIISWGLGCGQKDVPGVYTKVTNYLDWIRDNMRP

SEQ ID NO: 11 - protein, 5 aa, Protobothrops mucrosquamatus
KKKRT

SEQ ID NO: 12 - protein, 5 aa, Calloselasma rhodostoma
SRAGK

SEQ ID NO: 13 - protein, 5 aa, synthetic construct
IEEGT

SEQ ID NO: 14 - protein, 5 aa, synthetic construct
KKART

SEQ ID NO: 15 - protein, 5 aa, synthetic construct
MKKGT

SEQ ID NO: 16 - protein, 6 aa, synthetic construct
AKGDHP

SEQ ID NO: 17 - protein, 6 aa, synthetic construct
AKGDYP

SEQ ID NO: 18 - protein, 6 aa, synthetic construct
AKGDWP

SEQ ID NO: 19 - protein, 6 aa, synthetic construct
AKGDRP

SEQ ID NO: 20 - protein, 6 aa, synthetic construct
AKGDRR

SEQ ID NO: 21 - protein, 6 aa, synthetic construct
AKGDRK

SEQ ID NO: 22 - protein, 6 aa, synthetic construct
AKGDKR

SEQ ID NO: 23 - protein, 6 aa, synthetic construct
AKGDKK

SEQ ID NO: 24 - protein, 6 aa, synthetic construct
AKGDNP

SEQ ID NO: 25 - protein, 6 aa, synthetic construct
AKGDFP

SEQ ID NO: 26 - protein, 6 aa, synthetic construct
AKGDWN

SEQ ID NO: 27 - protein, 6 aa, synthetic construct
PKGDMP

SEQ ID NO: 28 - protein, 6 aa, synthetic construct
ARGDWN

SEQ ID NO: 29 - protein, 7 aa, Protobothrops mucrosquamatus
PRNGLYG

SEQ ID NO: 30 - protein, 4 aa, Calloselasma rhodostoma
PRYH

SEQ ID NO: 31 - protein, 7 aa, synthetic construct
PRNRLYG

SEQ ID NO: 32 - protein, 4 aa, synthetic construct
PRNS

SEQ ID NO: 33 - protein, 6 aa, synthetic construct
PRNRFH

SEQ ID NO: 34 - protein, 73 aa, synthetic construct
EAGEECDCGSPENPCCDAATCKLRPGAQCAEGLCCDQCRFKKKRTICRRAKGDRRDDRCTGQSADCPRNRLYG

SEQ ID NO: 35 - protein, 609 aa, synthetic construct
SYQVICRDEKTQMIYQQHQSWLRPVLRSNRVEYCWCNSGRAQCHSVPVKSCSEPRCFNGGTCQQALYFSDFVCQCPEGFAGKCCEIDTRATCYEDQGISYRGNWSTAESGAECTNWQSSALAQKPYSGRRPDAIRLGLGNHNYCRNPDRDSKPWCYVFKAGKYSSEFCSTPACSEGNSDCYFGNGSAYRGTHSLTESGASCLPWNSMILIGKVYTAQNPSAQALGLGKHNYCRNPDGDAKPWCHVLKNRRLTWEYCDVPSCSTCGLRQYSQPQFRIKGGLFADIASHPWQAAIFAAAAASPGERFLCGGILISSCWILSAAHCFQERFPPHHLTVILGRTYRVVPGEEEQKFEVEKYIVHKEFDDDTYDNDIALLQLKSDSSRCAQESSVVRTVCLPPADLQLPDWTECELSGYGKHEALSPFYSERLKEAHVRLYPSSRCTSQHLLNRTVTDNMLCAGDTRSGGPQANLHDACQGDSGGPLVCLNDGRMTLVGIISWGLGCGQKDVPGVYTKVTNYLDWIRDNMRPGGGGGGGGGEAGEECDCGSPENPCCDAATCKLRPGAQCAEGLCCDQCRFKKKRTICRRAKGDRRDDRCTGQSADCPRNRLYG

SEQ ID NO: 36 - protein, 615 aa, synthetic construct
SYQVICRDEKTQMIYQQHQSWLRPVLRSNRVEYCWCNSGRAQCHSVPVKSCSEPRCFNGGTCQQALYFSDFVCQCPEGFAGKCCEIDTRATCYEDQGISYRGNWSTAESGAECTNWQSSALAQKPYSGRRPDAIRLGLGNHNYCRNPDRDSKPWCYVFKAGKYSSEFCSTPACSEGNSDCYFGNGSAYRGTHSLTESGASCLPWNSMILIGKVYTAQNPSAQALGLGKHNYCRNPDGDAKPWCHVLKNRRLTWEYCDVPSCSTCGLRQYSQPQFRIKGGLFADIASHPWQAAIFAAAAASPGERFLCGGILISSCWILSAAHCFQERFPPHHLTVILGRTYRVVPGEEEQKFEVEKYIVHKEFDDDTYDNDIALLQLKSDSSRCAQESSVVRTVCLPPADLQLPDWTECELSGYGKHEALSPFYSERLKEAHVRLYPSSRCTSQHLLNRTVTDNMLCAGDTRSGGPQANLHDACQGDSGGPLVCLNDGRMTLVGIISWGLGCGQKDVPGVYTKVTNYLDWIRDNMRPGGGGSGGGGSGGGGSEAGEECDCGSPENPCCDAATCKLRPGAQCAEGLCCDQCRFKKKRTICRRAKGDRRDDRCTGQSADCPRNRLYG

SEQ ID NO: 37 - protein, 606 aa, synthetic construct
SYQVICRDEKTQMIYQQHQSWLRPVLRSNRVEYCWCNSGRAQCHSVPVKSCSEPRCFNGGTCQQALYFSDFVCQCPEGFAGKCCEIDTRATCYEDQGISYRGNWSTAESGAECTNWQSSALAQKPYSGRRPDAIRLGLGNHNYCRNPDRDSKPWCYVFKAGKYSSEFCSTPACSEGNSDCYFGNGSAYRGTHSLTESGASCLPWNSMILIGKVYTAQNPSAQALGLGKHNYCRNPDGDAKPWCHVLKNRRLTWEYCDVPSCSTCGLRQYSQPQFRIKGGLFADIASHPWQAAIFAAAAASPGERFLCGGILISSCWILSAAHCFQERFPPHHLTVILGRTYRVVPGEEEQKFEVEKYIVHKEFDDDTYDNDIALLQLKSDSSRCAQESSVVRTVCLPPADLQLPDWTECELSGYGKHEALSPFYSERLKEAHVRLYPSSRCTSQHLLNRTVTDNMLCAGDTRSGGPQANLHDACQGDSGGPLVCLNDGRMTLVGIISWGLGCGQKDVPGVYTKVTNYLDWIRDNMRPPAPAPAEAGEECDCGSPENPCCDAATCKLRPGAQCAEGLCCDQCRFKKKRTICRRAKGDRRDDRCTGQSADCPRNRLYG

SEQ ID NO: 38 - protein, 610 aa, synthetic construct
SYQVICRDEKTQMIYQQHQSWLRPVLRSNRVEYCWCNSGRAQCHSVPVKSCSEPRCFNGGTCQQALYFSDFVCQCPEGFAGKCCEIDTRATCYEDQGISYRGNWSTAESGAECTNWQSSALAQKPYSGRRPDAIRLGLGNHNYCRNPDRDSKPWCYVFKAGKYSSEFCSTPACSEGNSDCYFGNGSAYRGTHSLTESGASCLPWNSMILIGKVYTAQNPSAQALGLGKHNYCRNPDGDAKPWCHVLKNRRLTWEYCDVPSCSTCGLRQYSQPQFRIKGGLFADIASHPWQAAIFAAAAASPGERFLCGGILISSCWILSAAHCFQERFPPHHLTVILGRTYRVVPGEEEQKFEVEKYIVHKEFDDDTYDNDIALLQLKSDSSRCAQESSVVRTVCLPPADLQLPDWTECELSGYGKHEALSPFYSERLKEAHVRLYPSSRCTSQHLLNRTVTDNMLCAGDTRSGGPQANLHDACQGDSGGPLVCLNDGRMTLVGIISWGLGCGQKDVPGVYTKVTNYLDWIRDNMRPPAPAPAPAPAEAGEECDCGSPENPCCDAATCKLRPGAQCAEGLCCDQCRFKKKRTICRRAKGDRRDDRCTGQSADCPRNRLYG

SEQ ID NO: 39 - protein, 614 aa, synthetic construct
SYQVICRDEKTQMIYQQHQSWLRPVLRSNRVEYCWCNSGRAQCHSVPVKSCSEPRCFNGGTCQQALYFSDFVCQCPEGFAGKCCEIDTRATCYEDQGISYRGNWSTAESGAECTNWQSSALAQKPYSGRRPDAIRLGLGNHNYCRNPDRDSKPWCYVFKAGKYSSEFCSTPACSEGNSDCYFGNGSAYRGTHSLTESGASCLPWNSMILIGKVYTAQNPSAQALGLGKHNYCRNPDGDAKPWCHVLKNRRLTWEYCDVPSCSTCGLRQYSQPQFRIKGGLFADIASHPWQAAIFAAAAASPGERFLCGGILISSCWILSAAHCFQERFPPHHLTVILGRTYRVVPGEEEQKFEVEKYIVHKEFDDDTYDNDIALLQLKSDSSRCAQESSVVRTVCLPPADLQLPDWTECELSGYGKHEALSPFYSERLKEAHVRLYPSSRCTSQHLLNRTVTDNMLCAGDTRSGGPQANLHDACQGDSGGPLVCLNDGRMTLVGIISWGLGCGQKDVPGVYTKVTNYLDWIRDNMRPPAPAPAPAPAPAPAEAGEECDCGSPENPCCDAATCKLRPGAQCAEGLCCDQCRFKKKRTICRRAKGDRRDDRCTGQSADCPRNRLYG

SEQ ID NO: 40 - protein, 615 aa, synthetic construct
SYQVICRDEKTQMIYQQHQSWLRPVLRSNRVEYCWCNSGRAQCHSVPVKSCSEPRCFNGGTCQQALYFSDFVCQCPEGFAGKCCEIDTRATCYEDQGISYRGNWSTAESGAECTNWQSSALAQKPYSGRRPDAIRLGLGNHNYCRNPDRDSKPWCYVFKAGKYSSEFCSTPACSEGNSDCYFGNGSAYRGTHSLTESGASCLPWNSMILIGKVYTAQNPSAQALGLGKHNYCRNPDGDAKPWCHVLKNRRLTWEYCDVPSCSTCGLRQYSQPQFRIKGGLFADIASHPWQAAIFAAAAASPGERFLCGGILISSCWILSAAHCFQERFPPHHLTVILGRTYRVVPGEEEQKFEVEKYIVHKEFDDDTYDNDIALLQLKSDSSRCAQESSVVRTVCLPPADLQLPDWTECELSGYGKHEALSPFYSERLKEAHVRLYPSSRCTSQHLLNRTVTDNMLCAGDTRSGGPQANLHDACQGDSGGPLVCLNDGRMTLVGIISWGLGCGQKDVPGVYTKVTNYLDWIRDNMRPEAAAKGGGGSGGGGSEAGEECDCGSPENPCCDAATCKLRPGAQCAEGLCCDQCRFKKKRTICRRAKGDRRDDRCTGQSADCPRNRLYG

SEQ ID NO: 41 - protein, 615 aa, synthetic construct
SYQVICRDEKTQMIYQQHQSWLRPVLRSNRVEYCWCNSGRAQCHSVPVKSCSEPRCFNGGTCQQALYFSDFVCQCPEGFAGKCCEIDTRATCYEDQGISYRGNWSTAESGAECTNWQSSALAQKPYSGRRPDAIRLGLGNHNYCRNPDRDSKPWCYVFKAGKYSSEFCSTPACSEGNSDCYFGNGSAYRGTHSLTESGASCLPWNSMILIGKVYTAQNPSAQALGLGKHNYCRNPDGDAKPWCHVLKNRRLTWEYCDVPSCSTCGLRQYSQPQFRIKGGLFADIASHPWQAAIFAAAAASPGERFLCGGILISSCWILSAAHCFQERFPPHHLTVILGRTYRVVPGEEEQKFEVEKYIVHKEFDDDTYDNDIALLQLKSDSSRCAQESSVVRTVCLPPADLQLPDWTECELSGYGKHEALSPFYSERLKEAHVRLYPSSRCTSQHLLNRTVTDNMLCAGDTRSGGPQANLHDACQGDSGGPLVCLNDGRMTLVGIISWGLGCGQKDVPGVYTKVTNYLDWIRDNMRPEAAAKEAAAKEAAAKEAGEECDCGSPENPCCDAATCKLRPGAQCAEGLCCDQCRFKKKRTICRRAKGDRRDDRCTGQSADCPRNRLYG

SEQ ID NO: 42 - protein, 610 aa, synthetic construct
EAGEECDCGSPENPCCDAATCKLRPGAQCAEGLCCDQCRFKKKRTICRRAKGDRRDDRCTGQSADCPRNRLYGPAPAPAPAPASYQVICRDEKTQMIYQQHQSWLRPVLRSNRVEYCWCNSGRAQCHSVPVKSCSEPRCFNGGTCQQALYFSDFVCQCPEGFAGKCCEIDTRATCYEDQGISYRGNWSTAESGAECTNWQSSALAQKPYSGRRPDAIRLGLGNHNYCRNPDRDSKPWCYVFKAGKYSSEFCSTPACSEGNSDCYFGNGSAYRGTHSLTESGASCLPWNSMILIGKVYTAQNPSAQALGLGKHNYCRNPDGDAKPWCHVLKNRRLTWEYCDVPSCSTCGLRQYSQPQFRIKGGLFADIASHPWQAAIFAAAAASPGERFLCGGILISSCWILSAAHCFQERFPPHHLTVILGRTYRVVPGEEEQKFEVEKYIVHKEFDDDTYDNDIALLQLKSDSSRCAQESSVVRTVCLPPADLQLPDWTECELSGYGKHEALSPFYSERLKEAHVRLYPSSRCTSQHLLNRTVTDNMLCAGDTRSGGPQANLHDACQGDSGGPLVCLNDGRMTLVGIISWGLGCGQKDVPGVYTKVTNYLDWIRDNMRP